European Patent Specification EP 3 817 775 B1, published September 4, 2024. Title: IMPROVEMENTS IN IMMUNOGENIC CONJUGATES. Applicant: SUTROVAX, INC. The sequence listing filed with the application follows.

SEQUENCE LISTING (5 sequences)

SEQ ID NO: 1 - protein, 535 aa, Corynebacterium diphtheriae
GADDVVDSSKSFVMENFSSYHGTKPGYVDSIQKGIQKPKSGTQGNYDDDWKEFYSTDNKYDAAGYSVDNENPLSGKAGGVVKVTYPGLTKVLALKVDNAETIKKELGLSLTEPLMEQVGTEEFIKRFGDGASRVVLSLPFAEGSSSVEYINNWEQAKALSVELEINFETRGKRGQDAMYEYMAQACAGNRVRRSVGSSLSCINLDWDVIRDKTKTKIESLKEHGPIKNKMSESPNKTVSEEKAKQYLEEFHQTALEHPELSELKTVTGTNPVFAGANYAAWAVNVAQVIDSETADNLEKTTAALSILPGIGSVMGIADGAVHHNTEEIVAQSIALSSLMVAQAIPLVGELVDIGFAAYNFVESIINLFQVVHNSYNRPAYSPGHKTQPFLHDGYAVSWNTVEDSIIRTGFQGESGHDIKITAENTPLPIAGVLLPTIPGKLDVNKSKTHISVNGRKIRMRCRAIDGDVTFCRPKSPVYVGNGVHANLHVAFHRSSSEKIHSNEISSDSIGVLGYQKTVDHTKVNSKLSLFFEIKS

SEQ ID NO: 2 - protein, 535 aa, Artificial Sequence
  CRM197 with Arg-Asn substitution
GADDVVDSSKSFVMENFSSYHGTKPGYVDSIQKGIQKPKSGTQGNYDDDWKEFYSTDNKYDAAGYSVDNENPLSGKAGGVVKVTYPGLTKVLALKVDNAETIKKELGLSLTEPLMEQVGTEEFIKRFGDGASRVVLSLPFAEGSSSVEYINNWEQAKALSVELEINFETRGKRGQDAMYEYMAQACAGNRVRNSVGSSLSCINLDWDVIRDKTKTKIESLKEHGPIKNKMSESPNKTVSEEKAKQYLEEFHQTALEHPELSELKTVTGTNPVFAGANYAAWAVNVAQVIDSETADNLEKTTAALSILPGIGSVMGIADGAVHHNTEEIVAQSIALSSLMVAQAIPLVGELVDIGFAAYNFVESIINLFQVVHNSYNRPAYSPGHKTQPFLHDGYAVSWNTVEDSIIRTGFQGESGHDIKITAENTPLPIAGVLLPTIPGKLDVNKSKTHISVNGRKIRMRCRAIDGDVTFCRPKSPVYVGNGVHANLHVAFHRSSSEKIHSNEISSDSIGVLGYQKTVDHTKVNSKLSLFFEIKS

SEQ ID NO: 3 - protein, 536 aa, Artificial Sequence
  CRM197 with 6 preferred nnAA sites and N-terminus Met
  misc_feature (34)..(34): Xaa can be any non-naturally occurring amino acid
  misc_feature (213)..(213): Xaa can be any non-naturally occurring amino acid
  misc_feature (245)..(245): Xaa can be any non-naturally occurring amino acid
  misc_feature (265)..(265): Xaa can be any non-naturally occurring amino acid
  misc_feature (386)..(386): Xaa can be any non-naturally occurring amino acid
  misc_feature (527)..(527): Xaa can be any non-naturally occurring amino acid
MGADDVVDSSKSFVMENFSSYHGTKPGYVDSIQXGIQKPKSGTQGNYDDDWKEFYSTDNKYDAAGYSVDNENPLSGKAGGVVKVTYPGLTKVLALKVDNAETIKKELGLSLTEPLMEQVGTEEFIKRFGDGASRVVLSLPFAEGSSSVEYINNWEQAKALSVELEINFETRGKRGQDAMYEYMAQACAGNRVRRSVGSSLSCINLDWDVIRDXTKTKIESLKEHGPIKNKMSESPNKTVSEEKAXQYLEEFHQTALEHPELSELXTVTGTNPVFAGANYAAWAVNVAQVIDSETADNLEKTTAALSILPGIGSVMGIADGAVHHNTEEIVAQSIALSSLMVAQAIPLVGELVDIGFAAYNFVESIINLFQVVHNSYNRPAYSPGHXTQPFLHDGYAVSWNTVEDSIIRTGFQGESGHDIKITAENTPLPIAGVLLPTIPGKLDVNKSKTHISVNGRKIRMRCRAIDGDVTFCRPKSPVYVGNGVHANLHVAFHRSSSEKIHSNEISSDSIGVLGYQKTVDHTKVNSXLSLFFEIKS

SEQ ID NO: 4 - protein, 536 aa, Artificial Sequence
  CRM197 with Arg-Asn substitution, 6 preferred nnAA sites, and N-terminus Met
  misc_feature (34)..(34): Xaa can be any non-naturally occurring amino acid
  misc_feature (213)..(213): Xaa can be any non-naturally occurring amino acid
  misc_feature (245)..(245): Xaa can be any non-naturally occurring amino acid
  misc_feature (265)..(265): Xaa can be any non-naturally occurring amino acid
  misc_feature (386)..(386): Xaa can be any non-naturally occurring amino acid
  misc_feature (527)..(527): Xaa can be any non-naturally occurring amino acid
MGADDVVDSSKSFVMENFSSYHGTKPGYVDSIQXGIQKPKSGTQGNYDDDWKEFYSTDNKYDAAGYSVDNENPLSGKAGGVVKVTYPGLTKVLALKVDNAETIKKELGLSLTEPLMEQVGTEEFIKRFGDGASRVVLSLPFAEGSSSVEYINNWEQAKALSVELEINFETRGKRGQDAMYEYMAQACAGNRVRNSVGSSLSCINLDWDVIRDXTKTKIESLKEHGPIKNKMSESPNKTVSEEKAXQYLEEFHQTALEHPELSELXTVTGTNPVFAGANYAAWAVNVAQVIDSETADNLEKTTAALSILPGIGSVMGIADGAVHHNTEEIVAQSIALSSLMVAQAIPLVGELVDIGFAAYNFVESIINLFQVVHNSYNRPAYSPGHXTQPFLHDGYAVSWNTVEDSIIRTGFQGESGHDIKITAENTPLPIAGVLLPTIPGKLDVNKSKTHISVNGRKIRMRCRAIDGDVTFCRPKSPVYVGNGVHANLHVAFHRSSSEKIHSNEISSDSIGVLGYQKTVDHTKVNSXLSLFFEIKS

SEQ ID NO: 5 - protein, 346 aa, Haemophilus influenzae
CSSHSSNMANTQMKSDKIIIAHRGASGYLPEHTLESKALAFAQQADYLEQDLAMTKDGRLVVIHDHFLDGLTDVAKKFPHRHRKDGRYYVIDFTLKEIQSLEMTENFETKDGKQAQVYPNRFPLWKSHFRIHTFEDEIEFIQGLEKSTGKKVGIYPEIKAPWFHHQNGKDIAAETLKVLKKYGYDKKTDMVYLQTFDFNELKRIKTELLPQMGMDLKLVQLIAYTDWKETQEKDPKGYWVNYNYDWMFKPGAMAEVVKYADGVGPGWYMLVNKEESKPDNIVYTPLVKELAQYNVEVHPYTVRKDALPEFFTDVNQMYDALLNKSGATGVFTDFPDTGVEFLKGIK